European Patent Specification EP 3 587 445 B1, published December 13, 2023. Title: COMPOSITIONS, METHODS AND/OR KITS COMPRISING A RECOMBINANT HUMAN CD38-EXTRACELLULAR DOMAIN. Applicant: GRIFOLS DIAGNOSTIC SOLUTIONS INC. The sequence listing filed with the application follows.

SEQUENCE LISTING (30 sequences)

SEQ ID NO: 1 - protein, 257 aa, Synthetic
PRWRQQWSGPGTTKRFPETVLARCVKYTEIHPEMRHVDCQSVWDAFKGAFISKHPCNITEEDYQPLMKLGTQTVPCNKILLWSRIKDLAHQFTQVQRDMFTLEDTLLGYLADDLTWCGEFNTSKINYQSCPDWRKDCSNNPVSVFWKTVSRRFAEAACDVVHVMLNGSRSKIFDKNSTFGSVEVHNLQPEKVQTLEAWVIHGGREDSRDLCQDPTIKELESIISKRNIQFSCKNIYRPDKFLQCVKNPEDSSCTSEI

SEQ ID NO: 2 - protein, 51 aa, Synthetic
LQPEKVQTLEAWVIHGGREDSRDLCQDPTIKELESIISKRNIQFSCKNIYR

SEQ ID NO: 3 - protein, 12 aa, Synthetic
VQTLEAWVIHGG

SEQ ID NO: 4 - protein, 14 aa, Synthetic
SKRNIQFSCKNIYR

SEQ ID NO: 5 - protein, 239 aa, Synthetic
HGVPRDCGCKPCICTVPEVSSVFIFPPKPKDVLTITLTPKVTCVVVDISKDDPEVQFSWFVDDVEVHTAQTQPREEQFNSTFRSVSELPIMHQDWLNGKEFKCRVNSAAFPAPIEKTISKTKGRPKAPQVYTIPPPKEQMAKDKVSLTCMITDFFPEDITVEWQWNGQPAENYKNTQPIMDTDGSYFVYSKLNVQKSNWEAGNTFTCSVLHEGLHNHHTEKSLSHSPGIHHHHHHHHHH

SEQ ID NO: 6 - protein, 392 aa, Synthetic
MHHHHHHHHHHGSKTEEGKLVIWINGDKGYNGLAEVGKKFEKDTGIKVTVEHPDKLEEKFPQVAATGDGPDIIFWAHDRFGGYAQSGLLAEITPDKAFQDKLYPFTWDAVRYNGKLIAYPIAVEALSLIYNKDLLPNPPKTWEEIPALDKELKAKGKSALMFNLQEPYFTWPLIAADGGYAFKYENGKYDIKDVGVDNAGAKAGLTFLVDLIKNKHMNADTDYSIAEAAFNKGETAMTINGPWAWSNIDTSKVNYGVTVLPTFKGQPSKPFVGVLSAGINAASPNKELAKEFLENYLLTDEGLEAVNKDKPLGAVALKSYEEELAKDPRIAATMENAQKGEIMPNIPQMSAFWYAVRTAVINAASGRQTVDEALKDAQTNSSSGENLYFQGT

SEQ ID NO: 7 - protein, 498 aa, Synthetic
VDRWRQQWSGPGTTKRFPETVLARCVKYTEIHPEMRHVDCQSVWDAFKGAFISKHPCNITEEDYQPLMKLGTQTVPCNKILLWSRIKDLAHQFTQVQRDMFTLEDTLLGYLADDLTWCGEFNTSKINYQSCPDWRKDCSNNPVSVFWKTVSRRFAEAACDVVHVMLNGSRSKIFDKNSTFGSVEVHNLQPEKVQTLEAWVIHGGREDSRDLCQDPTIKELESIISKRNIQFSCKNIYRPDKFLQCVKNPEDSSCTSEIPPGVPRDCGCKPCICTVPEVSSVFIFPPKPKDVLTITLTPKVTCVVVDISKDDPEVQFSWFVDDVEVHTAQTQPREEQFNSTFRSVSELPIMHQDWLNGKEFKCRVNSAAFPAPIEKTISKTKGRPKAPQVYTIPPPKEQMAKDKVSLTCMITDFFPEDITVEWQWNGQPAENYKNTQPIMDTDGSYFVYSKLNVQKSNWEAGNTFTCSVLHEGLHNHHTEKSLSHSPGIHHHHHHHHHH

SEQ ID NO: 8 - protein, 270 aa, Synthetic
VDRWRQQWSGPGTTKRFPETVLARCVKYTEIHPEMRHVDCQSVWDAFKGAFISKHPCNITEEDYQPLMKLGTQTVPCNKILLWSRIKDLAHQFTQVQRDMFTLEDTLLGYLADDLTWCGEFNTSKINYQSCPDWRKDCSNNPVSVFWKTVSRRFAEAACDVVHVMLNGSRSKIFDKNSTFGSVEVHNLQPEKVQTLEAWVIHGGREDSRDLCQDPTIKELESIISKRNIQFSCKNIYRPDKFLQCVKNPEDSSCTSEIGIHHHHHHHHHH

SEQ ID NO: 9 - protein, 648 aa, Synthetic
MHHHHHHHHHHGSKTEEGKLVIWINGDKGYNGLAEVGKKFEKDTGIKVTVEHPDKLEEKFPQVAATGDGPDIIFWAHDRFGGYAQSGLLAEITPDKAFQDKLYPFTWDAVRYNGKLIAYPIAVEALSLIYNKDLLPNPPKTWEEIPALDKELKAKGKSALMFNLQEPYFTWPLIAADGGYAFKYENGKYDIKDVGVDNAGAKAGLTFLVDLIKNKHMNADTDYSIAEAAFNKGETAMTINGPWAWSNIDTSKVNYGVTVLPTFKGQPSKPFVGVLSAGINAASPNKELAKEFLENYLLTDEGLEAVNKDKPLGAVALKSYEEELAKDPRIAATMENAQKGEIMPNIPQMSAFWYAVRTAVINAASGRQTVDEALKDAQTNSSSGENLYFQGTRWRQQWSGPGTTKRFPETVLARCVKYTEIHPEMRHVDCQSVWDAFKGAFISKHPCNITEEDYQPLMKLGTQTVPCNKILLWSRIKDLAHQFTQVQRDMFTLEDTLLGYLADDLTWCGEFNTSKINYQSCPDWRKDCSNNPVSVFWKTVSRRFAEAACDVVHVMLNGSRSKIFDKNSTFGSVEVHNLQPEKVQTLEAWVIHGGREDSRDLCQDPTIKELESIISKRNIQFSCKNIYRPDKFLQCVKNPEDSSCTSEI

SEQ ID NO: 10 - protein, 278 aa, Synthetic
MHHHHHHHHHHGSGENLYFQGTRWRQQWSGPGTTKRFPETVLARCVKYTEIHPEMRHVDCQSVWDAFKGAFISKHPCNITEEDYQPLMKLGTQTVPCNKILLWSRIKDLAHQFTQVQRDMFTLEDTLLGYLADDLTWCGEFNTSKINYQSCPDWRKDCSNNPVSVFWKTVSRRFAEAACDVVHVMLNGSRSKIFDKNSTFGSVEVHNLQPEKVQTLEAWVIHGGREDSRDLCQDPTIKELESIISKRNIQFSCKNIYRPDKFLQCVKNPEDSSCTSEI

SEQ ID NO: 11 - protein, 443 aa, Synthetic
MHHHHHHHHHHGSKTEEGKLVIWINGDKGYNGLAEVGKKFEKDTGIKVTVEHPDKLEEKFPQVAATGDGPDIIFWAHDRFGGYAQSGLLAEITPDKAFQDKLYPFTWDAVRYNGKLIAYPIAVEALSLIYNKDLLPNPPKTWEEIPALDKELKAKGKSALMFNLQEPYFTWPLIAADGGYAFKYENGKYDIKDVGVDNAGAKAGLTFLVDLIKNKHMNADTDYSIAEAAFNKGETAMTINGPWAWSNIDTSKVNYGVTVLPTFKGQPSKPFVGVLSAGINAASPNKELAKEFLENYLLTDEGLEAVNKDKPLGAVALKSYEEELAKDPRIAATMENAQKGEIMPNIPQMSAFWYAVRTAVINAASGRQTVDEALKDAQTNSSSGENLYFQGTLQPEKVQTLEAWVIHGGREDSRDLCQDPTIKELESIISKRNIQFSCKNIYR

SEQ ID NO: 12 - protein, 497 aa, Synthetic
VDRWRQQWSGPGTTKRFPETVLARCVKYTEIHPEMRHVDCQSVWDAFKGAFISKHPCNITEEDYQPLMKLGTQTVPCNKILLWSRIKDLAHQFTQVQRDMFTLEDTLLGYLADDLTWCGEFNTSKINYQSCPDWRKDCSNNPVSVFWKTVSRRFAEAACDVVHVMLNGSRSKIFDKNSTFGSVEVHNLQPEKVQTLEAWVIHGGREDSRDLCQDPTIKELESIISKRNIQFSCKNIYRPDKFLQCVKNPEDSSCTSEIPPGGGGSGGGSGGGSVPEVSSVFIFPPKPKDVLTITLTPKVTCVVVDISKDDPEVQFSWFVDDVEVHTAQTQPREEQFNSTFRSVSELPIMHQDWLNGKEFKCRVNSAAFPAPIEKTISKTKGRPKAPQVYTIPPPKEQMAKDKVSLTCMITDFFPEDITVEWQWNGQPAENYKNTQPIMDTDGSYFVYSKLNVQKSNWEAGNTFTCSVLHEGLHNHHTEKSLSHSPGIHHHHHHHHHH

SEQ ID NO: 13 - protein, 488 aa, Synthetic
VDRWRQQWSGPGTTKRFPETVLARCVKYTEIHPEMRHVDCQSVWDAFKGAFISKHPCNITEEDYQPLMKLGTQTVPCNKILLWSRIKDLAHQFTQVQRDMFTLEDTLLGYLADDLTWCGEFNTSKINYQSCPDWRKDCSNNPVSVFWKTVSRRFAEAACDVVHVMLNGSRSKIFDKNSTFGSVEVHNLQPEKVQTLEAWVIHGGREDSRDLCQDPTIKELESIISKRNIQFSCKNIYRPDKFLQCVKNPEDSSCTSEIPPGVPRDCGCKPCICTVPEVSSVFIFPPKPKDVLTITLTPKVTCVVVDISKDDPEVQFSWFVDDVEVHTAQTQPREEQFNSTFRSVSELPIMHQDWLNGKEFKCRVNSAAFPAPIEKTISKTKGRPKAPQVYTIPPPKEQMAKDKVSLTCMITDFFPEDITVEWQWNGQPAENYKNTQPIMDTDGSYFVYSKLNVQKSNWEAGNTFTCSVLHEGLHNHHTEKSLSHSPGI

SEQ ID NO: 14 - protein, 281 aa, Synthetic
VDRWRQQWSGPGTTKRFPETVLARCVKYTEIHPEMRHVDCQSVWDAFKGAFISKHPCNITEEDYQPLMKLGTQTVPCNKILLWSRIKDLAHQFTQVQRDMFTLEDTLLGYLADDLTWCGEFNTSKINYQSCPDWRKDCSNNPVSVFWKTVSRRFAEAACDVVHVMLNGSRSKIFDKNSTFGSVEVHNLQPEKVQTLEAWVIHGGREDSRDLCQDPTIKELESIISKRNIQFSCKNIYRPDKFLQCVKNPEDSSCTSEIPPGGGGGSGGGGSHHHHHHHHHH

SEQ ID NO: 15 - protein, 252 aa, Synthetic
VDRSRIRTISARLEYTRPHRSDLPGVPRDCGCKPCICTVPEVSSVFIFPPKPKDVLTITLTPKVTCVVVDISKDDPEVQFSWFVDDVEVHTAQTQPREEQFNSTFRSVSELPIMHQDWLNGKEFKCRVNSAAFPAPIEKTISKTKGRPKAPQVYTIPPPKEQMAKDKVSLTCMITDFFPEDITVEWQWNGQPAENYKNTQPIMDTDGSYFVYSKLNVQKSNWEAGNTFTCSVLHEGLHNHHTEKSLSHSPGI

SEQ ID NO: 16 - protein, 262 aa, Synthetic
VDRSRIRTISARLEYTRPHRSDLPGVPRDCGCKPCICTVPEVSSVFIFPPKPKDVLTITLTPKVTCVVVDISKDDPEVQFSWFVDDVEVHTAQTQPREEQFNSTFRSVSELPIMHQDWLNGKEFKCRVNSAAFPAPIEKTISKTKGRPKAPQVYTIPPPKEQMAKDKVSLTCMITDFFPEDITVEWQWNGQPAENYKNTQPIMDTDGSYFVYSKLNVQKSNWEAGNTFTCSVLHEGLHNHHTEKSLSHSPGIHHHHHHHHHH

SEQ ID NO: 17 - protein, 261 aa, Synthetic
VDRSRIRTISARLEYTRPHRSDLPGGGGSGGGSGGGSVPEVSSVFIFPPKPKDVLTITLTPKVTCVVVDISKDDPEVQFSWFVDDVEVHTAQTQPREEQFNSTFRSVSELPIMHQDWLNGKEFKCRVNSAAFPAPIEKTISKTKGRPKAPQVYTIPPPKEQMAKDKVSLTCMITDFFPEDITVEWQWNGQPAENYKNTQPIMDTDGSYFVYSKLNVQKSNWEAGNTFTCSVLHEGLHNHHTEKSLSHSPGIHHHHHHHHHH

SEQ ID NO: 18 - protein, 236 aa, Synthetic
VPRDCGCKPCICTVPEVSSVFIFPPKPKDVLTITLTPKVTCVVVDISKDDPEVQFSWFVDDVEVHTAQTQPREEQFNSTFRSVSELPIMHQDWLNGKEFKCRVNSAAFPAPIEKTISKTKGRPKAPQVYTIPPPKEQMAKDKVSLTCMITDFFPEDITVEWQWNGQPAENYKNTQPIMDTDGSYFVYSKLNVQKSNWEAGNTFTCSVLHEGLHNHHTEKSLSHSPGIGHHHHHHHH

SEQ ID NO: 19 - protein, 421 aa, Synthetic
MHHHHHHHHHHGSKTEEGKLVIWINGDKGYNGLAEVGKKFEKDTGIKVTVEHPDKLEEKFPQVAATGDGPDIIFWAHDRFGGYAQSGLLAEITPDKAFQDKLYPFTWDAVRYNGKLIAYPIAVEALSLIYNKDLLPNPPKTWEEIPALDKELKAKGKSALMFNLQEPYFTWPLIAADGGYAFKYENGKYDIKDVGVDNAGAKAGLTFLVDLIKNKHMNADTDYSIAEAAFNKGETAMTINGPWAWSNIDTSKVNYGVTVLPTFKGQPSKPFVGVLSAGINAASPNKELAKEFLENYLLTDEGLEAVNKDKPLGAVALKSYEEELAKDPRIAATMENAQKGEIMPNIPQMSAFWYAVRTAVINAASGRQTVDEALKDAQTNSSSGENLYFQGTGTSNASRSAGSTPGSSGRTSPSPSLSLIS

SEQ ID NO: 20 - protein, 365 aa, Synthetic
VDQLLFNKTKSVEFTFCNDTVVIPCFVTNMEAQNTTEVYVKWKFKGRDIYTFDGALNKSTVPTDFSSAKIEVSQLLKGDASLKMDKSDAVSHTGNYTCEVTELTREGETIIELKYRVVSWFSPNEGPGVPRDCGCKPCICTVPEVSSVFIFPPKPKDVLTITLTPKVTCVVVDISKDDPEVQFSWFVDDVEVHTAQTQPREEQFNSTFRSVSELPIMHQDWLNGKEFKCRVNSAAFPAPIEKTISKTKGRPKAPQVYTIPPPKEQMAKDKVSLTCMITDFFPEDITVEWQWNGQPAENYKNTQPIMDTDGSYFVYSKLNVQKSNWEAGNTFTCSVLHEGLHNHHTEKSLSHSPGIHHHHHHHHHH

SEQ ID NO: 21 - protein, 526 aa, Synthetic
HPICEVSKVASHLEVNCDKRNLTALPPDLPKDTTILHLSENLLYTFSLATLMPYTRLTQLNLDRSELTKLQVDGTLPVLGTLDLSHNQLQSLPLLGQTLPALTVLDVSFNRLTSLPLGALRGLGELQELYLKGNELKTLPPGLLTPTPKLEKLSLANNNLTELPAGLLNGLENLDTLLLQENSLYTIPKGFFGSHLLPFAFLHGNPWLCNCEILYFRRWLQDNAENVYVWKQTVDVKAMTSNVASVQCDNSDKFPVYKYPGKGCPTLGDEGDTDLYDYYPEEDTEGDKVRVPRDCGCKPCICTVPEVSSVFIFPPKPKDVLTITLTPKVTCVVVDISKDDPEVQFSWFVDDVEVHTAQTQPREEQFNSTFRSVSELPIMHQDWLNGKEFKCRVNSAAFPAPIEKTISKTKGRPKAPQVYTIPPPKEQMAKDKVSLTCMITDFFPEDITVEWQWNGQPAENYKNTQPIMDTDGSYFVYSKLNVQKSNWEAGNTFTCSVLHEGLHNHHTEKSLSHSPGIGHHHHHHHH

SEQ ID NO: 22 - protein, 334 aa, Synthetic
HPICEVSKVASHLEVNCDKRNLTALPPDLPKDTTILHLSENLLYTFSLATLMPYTRLTQLNLDRSELTKLQVDGTLPVLGTLDLSHNQLQSLPLLGQTLPALTVLDVSFNRLTSLPLGALRGLGELQELYLKGNELKTLPPGLLTPTPKLEKLSLANNNLTELPAGLLNGLENLDTLLLQENSLYTIPKGFFGSHLLPFAFLHGNPWLCNCEILYFRRWLQDNAENVYVWKQTVDVKAMTSNVASVQCDNSDKFPVYKYPGKGCPTLGDEGDTDLYDYYPEEDTEGDKVRMDEKTTGWRGGHVVEGLAGELEQLRARLEHHPQGQREPHHHHHH

SEQ ID NO: 23 - protein, 296 aa, Synthetic
HPICEVSKVASHLEVNCDKRNLTALPPDLPKDTTILHLSENLLYTFSLATLMPYTRLTQLNLDRSELTKLQVDGTLPVLGTLDLSHNQLQSLPLLGQTLPALTVLDVSFNRLTSLPLGALRGLGELQELYLKGNELKTLPPGLLTPTPKLEKLSLANNNLTELPAGLLNGLENLDTLLLQENSLYTIPKGFFGSHLLPFAFLHGNPWLCNCEILYFRRWLQDNAENVYVWKQVVDVKAVTSNVASVQCDNSDKFPVYKYPGKGCPTLGDEGDTDLYDYYPEEDTEGDKVRHHHHHH

SEQ ID NO: 24 - protein, 336 aa, Synthetic
HPICEVSKVASHLEVNCDKRNLTALPPDLPKDTTILHLSENLLYTFSLATLMPYTRLTQLNLDRSELTKLQVDGTLPVLGTLDLSHNQLQSLPLLGQTLPALTVLDVSFNRLTSLPLGALRGLGELQELYLKGNELKTLPPGLLTPTPKLEKLSLANNNLTELPAGLLNGLENLDTLLLQENSLYTIPKGFFGSHLLPFAFLHGNPWLCNCEILYFRRWLQDNAENVYVWKQTVDVKAMTSNVASVQCDNSDKFPVYKYPGKGCPTLGDEGDTDLYDYYPEEDTEGDKVRKPLDGEYFTLQIRGRERFEMFRELNEALELKDAQAGKEPGHHHHHH

SEQ ID NO: 25 - protein, 123 aa, Synthetic
QLLFNKTKSVEFTFCNDTVVIPCFVTNMEAQNTTEVYVKWKFKGRDIYTFDGALNKSTVPTDFSSAKIEVSQLLKGDASLKMDKSDAVSHTGNYTCEVTELTREGETIIELKYRVVSWFSPNE

SEQ ID NO: 26 - protein, 290 aa, Synthetic
HPICEVSKVASHLEVNCDKRNLTALPPDLPKDTTILHLSENLLYTFSLATLMPYTRLTQLNLDRSELTKLQVDGTLPVLGTLDLSHNQLQSLPLLGQTLPALTVLDVSFNRLTSLPLGALRGLGELQELYLKGNELKTLPPGLLTPTPKLEKLSLANNNLTELPAGLLNGLENLDTLLLQENSLYTIPKGFFGSHLLPFAFLHGNPWLCNCEILYFRRWLQDNAENVYVWKQTVDVKAMTSNVASVQCDNSDKFPVYKYPGKGCPTLGDEGDTDLYDYYPEEDTEGDKVR

SEQ ID NO: 27 - protein, 290 aa, Synthetic
HPICEVSKVASHLEVNCDKRNLTALPPDLPKDTTILHLSENLLYTFSLATLMPYTRLTQLNLDRSELTKLQVDGTLPVLGTLDLSHNQLQSLPLLGQTLPALTVLDVSFNRLTSLPLGALRGLGELQELYLKGNELKTLPPGLLTPTPKLEKLSLANNNLTELPAGLLNGLENLDTLLLQENSLYTIPKGFFGSHLLPFAFLHGNPWLCNCEILYFRRWLQDNAENVYVWKQVVDVKAVTSNVASVQCDNSDKFPVYKYPGKGCPTLGDEGDTDLYDYYPEEDTEGDKVR

SEQ ID NO: 28 - protein, 11 aa, Synthetic
GGGGGSGGGGS

SEQ ID NO: 29 - protein, 13 aa, Synthetic
GGGGSGGGSGGGS

SEQ ID NO: 30 - protein, 13 aa, Synthetic
VPRDCGCKPCICT